European Patent Specification EP 3 778 901 B1, published May 6, 2026. Title: A novel promoter and preparation method of L-amino acid using thereof. Applicant: CJ CheilJedang Corporation. The sequence listing filed with the application follows.

SEQUENCE LISTING (16 sequences)

SEQ ID NO: 1 - DNA, 65 bp, Corynebacterium glutamicum
aattattcgactaatatcctcccccaaacacacattgataactgttgtgtggaagaatgtaccga

SEQ ID NO: 2 - DNA, 65 bp, Artificial Sequence
  hisEG promoter
aattattcgactaatatcctcccccaaacacacattgataactgttgtgtggtataatgtaccga

SEQ ID NO: 3 - DNA, 65 bp, Artificial Sequence
  hisEG promoter
aattattcgactaatatcctcccccaaacacacattgataactgttgtgtggtataatggaccga

SEQ ID NO: 4 - DNA, 75 bp, Artificial Sequence
  oligonucleotide
tcgtacagcgagtcaaatgtcttcactcggtacattataccacacaacagttatcaatgtgtgtttgggggagga

SEQ ID NO: 5 - DNA, 75 bp, Artificial Sequence
  oligonucleotide
tcgtacagcgagtcaaatgtcttcactcggtccattataccacacaacagttatcaatgtgtgtttgggggagga

SEQ ID NO: 6 - DNA, 33 bp, Artificial Sequence
  hisE-pro-2mt-AF
gatcctctagagtcgacttcgacgaatccctcg

SEQ ID NO: 7 - DNA, 32 bp, Artificial Sequence
  hisE-pro-2mt-AR
cggtacattataccacacaacagttatcaatg

SEQ ID NO: 8 - DNA, 32 bp, Artificial Sequence
  hisE-pro-2mt-BF
gtggtataatgtaccgagtgaagacatttgac

SEQ ID NO: 9 - DNA, 32 bp, Artificial Sequence
  hisE-pro-2mt-BR
atgcctgcaggtcgactgatacccaaatcgag

SEQ ID NO: 10 - DNA, 32 bp, Artificial Sequence
  hisE-pro-3mt-AR
cggtccattataccacacaacagttatcaatg

SEQ ID NO: 11 - DNA, 32 bp, Artificial Sequence
  hisE-pro-3mt-BF
gtggtataatggaccgagtgaagacatttgac

SEQ ID NO: 12 - DNA, 34 bp, Artificial Sequence
  hisG(G233H/T235Q)-AF
gatcctctagagtcgaccccaaacaagggctcgc

SEQ ID NO: 13 - DNA, 28 bp, Artificial Sequence
  hisG(G233H/T235Q)-AR
cgtgccagtggggatacctgtgggtggg

SEQ ID NO: 14 - DNA, 30 bp, Artificial Sequence
  hisG(G233H/T235Q)-BF
aaccccaggcctatcccacccacaggtatc

SEQ ID NO: 15 - DNA, 33 bp, Artificial Sequence
  hisG(G233H/T235Q)-BR
atgcctgcaggtcgacgcaaggttggcaacaac

SEQ ID NO: 16 - protein, 281 aa, Corynebacterium glutamicum [sequence omitted]